European Patent Application EP 4 491 718 A2, published January 15, 2025. Title: IL-13 RECEPTOR ALPHA 2 TARGETED, ZETAKINE DIRECTED T CELL IMMUNOTHERAPY. Applicant: Seattle Children's Hospital d/b/a Seattle Children's Research Institute. The sequence listing filed with the application follows.

SEQUENCE LISTING (27 sequences)

SEQ ID NO: 1 - protein, 15 aa, Homo sapiens
EPKSCDKTHTCPPCP

SEQ ID NO: 2 - protein, 12 aa, Homo sapiens
ERKCCVECPPCP

SEQ ID NO: 3 - protein, 61 aa, Homo sapiens
ELKTPLGDTHTCPRCPEPKSCDTPPPCPRCPEPKSCDTPPPCPRCPEPKSCDTPPPCPRCP

SEQ ID NO: 4 - protein, 12 aa, Homo sapiens
ESKYGPPCPSCP

SEQ ID NO: 5 - protein, 12 aa, synthetic construct
ESKYGPPCPPCP

SEQ ID NO: 6 - protein, 9 aa, synthetic construct
YGPPCPPCP

SEQ ID NO: 7 - protein, 10 aa, synthetic construct
KYGPPCPPCP

SEQ ID NO: 8 - protein, 13 aa, synthetic construct
EVVKYGPPCPPCP

SEQ ID NO: 9 - protein, 12 aa, synthetic construct
ESKYGPPCPPCP

SEQ ID NO: 10 - protein, 119 aa, synthetic construct
ESKYGPPCPPCPGQPREPQVYTLPPSQEEMTKNQVSLTCLVKGFYPSDIAVEWESNGQPENNYKTTPPVLDSDGSFFLYSRLTVDKSRWQEGNVFSCSVMHEALHNHYTQKSLSLSLGK

SEQ ID NO: 11 - protein, 229 aa, synthetic construct
ESKYGPPCPPCPAPEFLGGPSVFLFPPKPKDTLMISRTPEVTCVVVDVSQEDPEVQFNWYVDGVEVHNAKTKPREEQFNSTYRVVSVLTVLHQDWLNGKEYKCKVSNKGLPSSIEKTISKAKGQPREPQVYTLPPSQEEMTKNQVSLTCLVKGFYPSDIAVEWESNGQPENNYKTTPPVLDSDGSFFLYSRLTVDKSRWQEGNVFSCSVMHEALHNHYTQKSLSLSLGK

SEQ ID NO: 12 - DNA, 8740 bp, synthetic construct
  source 1..8740: mol_type = other DNA
gttagaccagatctgagcctgggagctctctggctaactagggaacccactgcttaagcctcaataaagcttgccttgagtgcttcaagtagtgtgtgcccgtctgttgtgtgactctggtaactagagatccctcagacccttttagtcagtgtggaaaatctctagcagtggcgcccgaacagggacttgaaagcgaaagggaaaccagaggagctctctcgacgcaggactcggcttgctgaagcgcgcacggcaagaggcgaggggcggcgactggtgagtacgccaaaaattttgactagcggaggctagaaggagagagatgggtgcgagagcgtcagtattaagcgggggagaattagatcgatgggaaaaaattcggttaaggccagggggaaagaaaaaatataaattaaaacatatagtatgggcaagcagggagctagaacgattcgcagttaatcctggcctgttagaaacatcagaaggctgtagacaaatactgggacagctacaaccatcccttcagacaggatcagaagaacttagatcattatataatacagtagcaaccctctattgtgtgcatcaaaggatagagataaaagacaccaaggaagctttagacaagatagaggaagagcaaaacaaaagtaagaaaaaagcacagcaagcagcagctgacacaggacacagcaatcaggtcagccaaaattaccctatagtgcagaacatccaggggcaaatggtacatcaggccatatcacctagaactttaaatgcatgggtaaaagtagtagaagagaaggctttcagcccagaagtgatacccatgttttcagcattatcagaaggagccaccccacaagatttaaacaccatgctaaacacagtggggggacatcaagcagccatgcaaatgttaaaagagaccatcaatgaggaagctgcaggcaaagagaagagtggtgcagagagaaaaaagagcagtgggaataggagctttgttccttgggttcttgggagcagcaggaagcactatgggcgcagcgtcaatgacgctgacggtacaggccagacaattattgtctggtatagtgcagcagcagaacaatttgctgagggctattgaggcgcaacagcatctgttgcaactcacagtctggggcatcaagcagctccaggcaagaatcctggctgtggaaagatacctaaaggatcaacagctcctggggatttggggttgctctggaaaactcatttgcaccactgctgtgccttggatctacaaatggcagtattcatccacaattttaaaagaaaaggggggattggggggtacagtgcaggggaaagaatagtagacataatagcaacagacatacaaactaaagaattacaaaaacaaattacaaaaattcaaaattttcgggtttattacagggacagcagagatccagtttggggatcaattgcatgaagaatctgcttagggttaggcgttttgcgctgcttcgcgaggatctgcgatcgctccggtgcccgtcagtgggcagagcgcacatcgcccacagtccccgagaagttggggggaggggtcggcaattgaaccggtgcctagagaaggtggcgcggggtaaactgggaaagtgatgtcgtgtactggctccgcctttttcccgagggtgggggagaaccgtatataagtgcagtagtcgccgtgaacgttctttttcgcaacgggtttgccgccagaacacagctgggctagcgtttaaacgggccctctagagccgccaccatgcttctcctggtgacaagccttctgctctgtgagttaccacacccagcattcctcctgatcccaggccctgtgcctccctctacagccctcaggtacctcattgaggagctggtcaacatcacccagaaccagaaggctccgctctgcaatggcagcatggtatggagcatcaacctgacagctggcatgtactgtgcagccctggaatccctgatcaacgtgtcaggctgcagtgccatcgagaagacccagaggatgctgagcggattctgcccgcacaaggtctcagctgggcagttttccagcttgcatgtccgagacaccaaaatcgaggtggcccagtttgtaaaggacctgctcttacatttaaagaaactttttcgcgagggacggttcaagaatctaagtaccggaccgccctgccccccttgccctggccagcctagagaaccccaggtgtacaccctgcctcccagccaggaagagatgaccaagaaccaggtgtccctgacctgcctggtcaaaggcttctaccccagcgatatcgccgtggaatgggagagcaacggccagcccgagaacaactacaagaccaccccccctgtgctggacagcgacggcagcttcttcctgtactcccggctgaccgtggacaagagccggtggcaggaaggcaacgtcttcagctgcagcgtgatgcacgaggccctgcacaaccactacacccagaagtccctgagcctgagcctgggcaagatgttctgggtgctggtggtggtcggaggcgtgctggcctgctacagcctgctggtcaccgtggccttcatcatcttttgggtgaaacggggcagaaagaaactcctgtatatattcaaacaaccatttatgagaccagtacaaactactcaagaggaagatggctgtagctgccgatttccagaagaagaagaaggaggatgtgaactgcgggtgaagttcagcagaagcgccgacgcccctgcctaccagcagggccagaatcagctgtacaacgagctgaacctgggcagaagggaagagtacgacgtcctggataagcggagaggccgggaccctgagatgggcggcaagcctcggcggaagaacccccaggaaggcctgtataacgaactgcagaaagacaagatggccgaggcctacagcgagatcggcatgaagggcgagcggaggcggggcaagggccacgacggcctgtatcagggcctgtccaccgccaccaaggatacctacgacgccctgcacatgcaggccctgcccccaaggctcgagggcggcggagagggcagaggaagtcttctaacatgcggtgacgtggaggagaatcccggccctaggatgcttctcctggtgacaagccttctgctctgtgagttaccacacccagcattcctcctgatcccacgcaaagtgtgtaacggaataggtattggtgaatttaaagactcactctccataaatgctacgaatattaaacacttcaaaaactgcacctccatcagtggcgatctccacatcctgccggtggcatttaggggtgactccttcacacatactcctcctctggatccacaggaactggatattctgaaaaccgtaaaggaaatcacagggtttttgctgattcaggcttggcctgaaaacaggacggacctccatgcctttgagaacctagaaatcatacgcggcaggaccaagcaacatggtcagttttctcttgcagtcgtcagcctgaacataacatccttgggattacgctccctcaaggagataagtgatggagatgtgataatttcaggaaacaaaaatttgtgctatgcaaatacaataaactggaaaaaactgtttgggacctccggtcagaaaaccaaaattataagcaacagaggtgaaaacagctgcaaggccacaggccaggtctgccatgccttgtgctcccccgagggctgctggggcccggagcccagggactgcgtctcttgccggaatgtcagccgaggcagggaatgcgtggacaagtgcaaccttctggagggtgagccaagggagtttgtggagaactctgagtgcatacagtgccacccagagtgcctgcctcaggccatgaacatcacctgcacaggacggggaccagacaactgtatccagtgtgcccactacattgacggcccccactgcgtcaagacctgcccggcaggagtcatgggagaaaacaacaccctggtctggaagtacgcagacgccggccatgtgtgccacctgtgccatccaaactgcacctacggatgcactgggccaggtcttgaaggctgtccaacgaatgggcctaagatcccgtccatcgccactgggatggtgggggccctcctcttgctgctggtggtggccctggggatcggcctcttcatgtgagcggccgctctagacccgggctgcaggaattcgatatcaagcttatcgataatcaacctctggattacaaaatttgtgaaagattgactggtattcttaactatgttgctccttttacgctatgtggatacgctgctttaatgcctttgtatcatgctattgcttcccgtatggctttcattttctcctccttgtataaatcctggttgctgtctctttatgaggagttgtggcccgttgtcaggcaacgtggcgtggtgtgcactgtgtttgctgacgcaacccccactggttggggcattgccaccacctgtcagctcctttccgggactttcgctttccccctccctattgccacggcggaactcatcgccgcctgccttgcccgctgctggacaggggctcggctgttgggcactgacaattccgtggtgttgtcggggaaatcatcgtcctttccttggctgctcgcctgtgttgccacctggattctgcgcgggacgtccttctgctacgtcccttcggccctcaatccagcggaccttccttcccgcggcctgctgccggctctgcggcctcttccgcgtcttcgccttcgccctcagacgagtcggatctccctttgggccgcctccccgcatcgataccgtcgactagccgtacctttaagaccaatgacttacaaggcagctgtagatcttagccactttttaaaagaaaaggggggactggaagggctaattcactcccaaagaagacaagatctgctttttgcctgtactgggtctctctggttagaccagatctgagcctgggagctctctggctaactagggaacccactgcttaagcctcaataaagcttgccttgagtgcttcaagtagtgtgtgcccgtctgttgtgtgactctggtaactagagatccctcagacccttttagtcagtgtggaaaatctctagcagaattcgatatcaagcttatcgataccgtcgacctcgagggggggcccggtaccgagctcggatccactagtccagtgtggtggaattctgcagatatccagcacagtggcggccactcaagtctggagggcacgttaaaacccgctgatcagcctcgactgtgccttctagttgccagccatctgttgtttgcccctcccccgtgccttccttgaccctggaaggtgccactcccactgtcctttcctaataaaatgaggaaattgcatcgcattgtctgagtaggtgtcattctattctggggggtggggtggggcaggacagcaagggggaggattgggaagacaatagcaggcatgctggggatgcggtgggctctatggcttctactgggcggttttatggacagcaagcgaaccggaattgccagctggggcgccctctggtaaggttgggaagccctgcaaagtaaactggatggctttctcgccgccaaggatctgatggcgcaggggatcaagctctgatcaagagacaggatgaggatcgtttcgcatgattgaacaagatggattgcacgcaggttctccggccgcttgggtggagaggctattcggctatgactgggcacaacagacaatcggctgctctgatgccgccgtgttccggctgtcagcgcaggggcgcccggttctttttgtcaagaccgacctgtccggtgccctgaatgaactgcaagacgaggcagcgcggctatcgtggctggccacgacgggcgttccttgcgcagctgtgctcgacgttgtcactgaagcgggaagggactggctgctattgggcgaagtgccggggcaggatctcctgtcatctcaccttgctcctgccgagaaagtatccatcatggctgatgcaatgcggcggctgcatacgcttgatccggctacctgcccattcgaccaccaagcgaaacatcgcatcgagcgagcacgtactcggatggaagccggtcttgtcgatcaggatgatctggacgaagagcatcaggggctcgcgccagccgaactgttcgccaggctcaaggcgagcatgcccgacggcgaggatctcgtcgtgacccatggcgatgcctgcttgccgaatatcatggtggaaaatggccgcttttctggattcatcgactgtggccggctgggtgtggcagaccgctatcaggacatagcgttggctacccgtgatattgctgaagagcttggcggcgaatgggctgaccgcttcctcgtgctttacggtatcgccgctcccgattcgcagcgcatcgccttctatcgccttcttgacgagttcttctgaattattaacgcttacaatttcctgatgcggtattttctccttacgcatctgtgcggtatttcacaccgcatacaggtggcacttttcggggaaatgtgcgcggaacccctatttgtttatttttctaaatacattcaaatatgtatccgctcatgaccaaaatcccttaacgtgagttttcgttccactgagcgtcagaccccgtagaaaagatcaaaggatcttcttgagatcctttttttctgcgcgtaatctgctgcttgcaaacaaaaaaaccaccgctaccagcggtggtttgtttgccggatcaagagctaccaactctttttccgaaggtaactggcttcagcagagcgcagataccaaatactgttcttctagtgtagccgtagttaggccaccacttcaagaactctgtagcaccgcctacatacctcgctctgctaatcctgttaccagtggctgctgccagtggcgataagtcgtgtcttaccgggttggactcaagacgatagttaccggataaggcgcagcggtcgggctgaacggggggttcgtgcacacagcccagcttggagcgaacgacctacaccgaactgagatacctacagcgtgagctatgagaaagcgccacgcttcccgaagggagaaaggcggacaggtatccggtaagcggcagggtcggaacaggagagcgcacgagggagcttccagggggaaacgcctggtatctttatagtcctgtcgggtttcgccacctctgacttgagcgtcgatttttgtgatgctcgtcaggggggcggagcctatggaaaaacgccagcaacgcggcctttttacggttcctggccttttgctggccttttgctcacatgttctttcctgcgttatcccctgattctgtggataaccgtattaccgcctttgagtgagctgataccgctcgccgcagccgaacgaccgagcgcagcgagtcagtgagcgaggaagcggaagagcgcccaatacgcaaaccgcctctccccgcgcgttggccgattcattaatgcagctggcacgacaggtttcccgactggaaagcgggcagtgagcgcaacgcaattaatgtgagttagctcactcattaggcaccccaggctttacactttatgcttccggctcgtatgttgtgtggaattgtgagcggataacaatttcacacaggaaacagctatgaccatgattacgccaagctcgaaattaaccctcactaaagggaacaaaagctggagctccaccgcggtggcggcctcgaggtcgagatccggtcgaccagcaaccatagtcccgcccctaactccgcccatcccgcccctaactccgcccagttccgcccattctccgccccatggctgactaattttttttatttatgcagaggccgaggccgcctcggcctctgagctattccagaagtagtgaggaggcttttttggaggcctaggcttttgcaaaaagcttcgacggtatcgattggctcatgtccaacattaccgccatgttgacattgattattgactagttattaatagtaatcaattacggggtcattagttcatagcccatatatggagttccgcgttacataacttacggtaaatggcccgcctggctgaccgcccaacgacccccgcccattgacgtcaataatgacgtatgttcccatagtaacgccaatagggactttccattgacgtcaatgggtggagtatttacggtaaactgcccacttggcagtacatcaagtgtatcatatgccaagtacgccccctattgacgtcaatgacggtaaatggcccgcctggcattatgcccagtacatgaccttatgggactttcctacttggcagtacatctacgtattagtcatcgctattaccatggtgatgcggttttggcagtacatcaatgggcgtggatagcggtttgactcacggggatttccaagtctccaccccattgacgtcaatgggagtttgttttggcaccaaaatcaacgggactttccaaaatgtcgtaacaactccgccccattgacgcaaatgggcggtaggcgtgtacggaattcggagtggcgagccctcagatcctgcatataagcagctgctttttgcctgtactgggtctctctg

SEQ ID NO: 13 - DNA, 8740 bp, synthetic construct; identical to SEQ ID NO: 12
  source 1..8740: mol_type = other DNA

SEQ ID NO: 14 - protein, 187 aa, synthetic construct
MVGSLNCIVAVSQNMGIGKNGDFPWPPLRNESRYFQRMTTTSSVEGKQNLVIMGKKTWFSIPEKNRPLKGRINLVLSRELKEPPQGAHFLSRSLDDALKLTEQPELANKVDMVWIVGGSSVYKEAMNHPGHLKLFVTRIMQDFESDTFFPEIDLEKYKLLPEYPGVLSDVQEEKGIKYKFEVYEKND

SEQ ID NO: 15 - DNA, 564 bp, synthetic construct
  source 1..564: mol_type = other DNA
atggttggttcgctaaactgcatcgtcgctgtgtcccagaacatgggcatcggcaagaacggggacttcccctggccaccgctcaggaatgaatccagatatttccagagaatgaccacaacctcttcagtagaaggtaaacagaatctggtgattatgggtaagaagacctggttctccattcctgagaagaatcgacctttaaagggtagaattaatttagttctcagcagagaactcaaggaacctccacaaggagctcattttctttccagaagtctagatgatgccttaaaacttactgaacaaccagaattagcaaataaagtagacatggtctggatagttggtggcagttctgtttataaggaagccatgaatcacccaggccatcttaaactatttgtgacaaggatcatgcaagactttgaaagtgacacgttttttccagaaattgatttggagaaatataaacttctgccagaatacccaggtgttctctctgatgtccaggaggagaaaggcattaagtacaaatttgaagtatatgagaagaatgattaa

SEQ ID NO: 16 - DNA, 402 bp, synthetic construct
  source 1..402: mol_type = other DNA
atgcttctcctggtgacaagccttctgctctgtgagttaccacacccagcattcctcctgatcccaggccctgtgcctccctctacagccctcaggtacctcattgaggagctggtcaacatcacccagaaccagaaggctccgctctgcaatggcagcatggtatggagcatcaacctgacagctggcatgtactgtgcagccctggaatccctgatcaacgtgtcaggctgcagtgccatcgagaagacccagaggatgctgagcggattctgcccgcacaaggtctcagctgggcagttttccagcttgcatgtccgagacaccaaaatcgaggtggcccagtttgtaaaggacctgctcttacatttaaagaaactttttcgcgagggacggttcaag

SEQ ID NO: 17 - protein, 134 aa, synthetic construct
MLLLVTSLLLCELPHPAFLLIPGPVPPSTALRYLIEELVNITQNQKAPLCNGSMVWSINLTAGMYCAALESLINVSGCSAIEKTQRMLSGFCPHKVSAGQFSSLHVRDTKIEVAQFVKDLLLHLKKLFREGRFK

SEQ ID NO: 18 - protein, 28 aa, Homo sapiens
MFWVLVVVGGVLACYSLLVTVAFIIFWV

SEQ ID NO: 19 - DNA, 66 bp, Homo sapiens
  source 1..66: mol_type = genomic DNA
atgcttctcctggtgacaagccttctgctctgtgagttaccacacccagcattcctcctgatccca

SEQ ID NO: 20 - DNA, 84 bp, Homo sapiens
  source 1..84: mol_type = genomic DNA
atgttctgggtgctggtggtggtcggaggcgtgctggcctgctacagcctgctggtcaccgtggccttcatcatcttttgggtg

SEQ ID NO: 21 - DNA, 126 bp, Homo sapiens
  source 1..126: mol_type = genomic DNA
aaacggggcagaaagaaactcctgtatatattcaaacaaccatttatgagaccagtacaaactactcaagaggaagatggctgtagctgccgatttccagaagaagaagaaggaggatgtgaactg

SEQ ID NO: 22 - DNA, 336 bp, Homo sapiens
  source 1..336: mol_type = genomic DNA
cgggtgaagttcagcagaagcgccgacgcccctgcctaccagcagggccagaatcagctgtacaacgagctgaacctgggcagaagggaagagtacgacgtcctggataagcggagaggccgggaccctgagatgggcggcaagcctcggcggaagaacccccaggaaggcctgtataacgaactgcagaaagacaagatggccgaggcctacagcgagatcggcatgaagggcgagcggaggcggggcaagggccacgacggcctgtatcagggcctgtccaccgccaccaaggatacctacgacgccctgcacatgcaggccctgcccccaagg

SEQ ID NO: 23 - DNA, 72 bp, synthetic construct
  source 1..72: mol_type = other DNA
ctcgagggcggcggagagggcagaggaagtcttctaacatgcggtgacgtggaggagaatcccggccctagg

SEQ ID NO: 24 - DNA, 1005 bp, synthetic construct
  source 1..1005: mol_type = other DNA
cgcaaagtgtgtaacggaataggtattggtgaatttaaagactcactctccataaatgctacgaatattaaacacttcaaaaactgcacctccatcagtggcgatctccacatcctgccggtggcatttaggggtgactccttcacacatactcctcctctggatccacaggaactggatattctgaaaaccgtaaaggaaatcacagggtttttgctgattcaggcttggcctgaaaacaggacggacctccatgcctttgagaacctagaaatcatacgcggcaggaccaagcaacatggtcagttttctcttgcagtcgtcagcctgaacataacatccttgggattacgctccctcaaggagataagtgatggagatgtgataatttcaggaaacaaaaatttgtgctatgcaaatacaataaactggaaaaaactgtttgggacctccggtcagaaaaccaaaattataagcaacagaggtgaaaacagctgcaaggccacaggccaggtctgccatgccttgtgctcccccgagggctgctggggcccggagcccagggactgcgtctcttgccggaatgtcagccgaggcagggaatgcgtggacaagtgcaaccttctggagggtgagccaagggagtttgtggagaactctgagtgcatacagtgccacccagagtgcctgcctcaggccatgaacatcacctgcacaggacggggaccagacaactgtatccagtgtgcccactacattgacggcccccactgcgtcaagacctgcccggcaggagtcatgggagaaaacaacaccctggtctggaagtacgcagacgccggccatgtgtgccacctgtgccatccaaactgcacctacggatgcactgggccaggtcttgaaggctgtccaacgaatgggcctaagatcccgtccatcgccactgggatggtgggggccctcctcttgctgctggtggtggccctggggatcggcctcttcatg

SEQ ID NO: 25 - DNA, 36 bp, synthetic construct
  source 1..36: mol_type = other DNA
gaatctaagtacggaccgccctgccccccttgccct

SEQ ID NO: 26 - DNA, 357 bp, synthetic construct
  source 1..357: mol_type = other DNA
gaatctaagtacggaccgccctgccccccttgccctggccagcctagagaaccccaggtgtacaccctgcctcccagccaggaagagatgaccaagaaccaggtgtccctgacctgcctggtcaaaggcttctaccccagcgatatcgccgtggaatgggagagcaacggccagcccgagaacaactacaagaccaccccccctgtgctggacagcgacggcagcttcttcctgtactcccggctgaccgtggacaagagccggtggcaggaaggcaacgtcttcagctgcagcgtgatgcacgaggccctgcacaaccactacacccagaagtccctgagcctgagcctgggcaag

SEQ ID NO: 27 - DNA, 685 bp, synthetic construct
  source 1..685: mol_type = other DNA
atctaagtacggaccgccctgccccccttgccctgcccccgagttcgacggcggacccagcgtgttcctgttcccccccaagcccaaggacaccctgatgatcagccggacccccgaggtgacctgcgtggtggtggacgtgagccaggaagatcccgaggtccagttcaattggtacgtggacggcgtggaagtgcacaacgccaagaccaagcccagagaggaacagttccagagcacctaccgggtggtgtctgtgctgaccgtgctgcaccaggactggctgaacggcaaagaatacaagtgcaaggtgtccaacaagggcctgcccagcagcatcgaaaagaccatcagcaaggccaagggccagcctcgcgagccccaggtgtacaccctgcctccctcccaggaagagatgaccaagaaccaggtgtccctgacctgcctggtgaagggcttctaccccagcgacatcgccgtggagtgggagagcaacggccagcctgagaacaactacaagaccacccctcccgtgctggacagcgacggcagcttcttcctgtacagccggctgaccgtggacaagagccggtggcaggaaggcaacgtctttagctgcagcgtgatgcacgaggccctgcacaaccactacacccagaagagcctgagcctgtccctgggcaag